European Patent Application EP 4 700 040 A1, published February 25, 2026. Title: PEPTIDE AND LUMINESCENT COMPLEX CONTANINING SAME. Applicant: Shenzhen Loggene Life Science & Technology Co.,Ltd. The sequence listing filed with the application follows.

SEQUENCE LISTING (106 sequences)

SEQ ID NO: 1 - protein, 11 aa, synthetic construct
VEGYRLFDKKW

SEQ ID NO: 2 - protein, 11 aa, synthetic construct
VDGWRLHEKIS

SEQ ID NO: 3 - protein, 11 aa, synthetic construct
VEGYRLFDRKS

SEQ ID NO: 4 - protein, 11 aa, synthetic construct
VEGWRLHEKIS

SEQ ID NO: 5 - protein, 11 aa, synthetic construct
VEGYRLHEKIS

SEQ ID NO: 6 - protein, 11 aa, synthetic construct
VEGYRLFDRKW

SEQ ID NO: 7 - protein, 11 aa, synthetic construct
VEGYRLFDRKL

SEQ ID NO: 8 - protein, 11 aa, synthetic construct
VEGYRLFKREL

SEQ ID NO: 9 - protein, 11 aa, synthetic construct
VEGYRLFDRVW

SEQ ID NO: 10 - protein, 11 aa, synthetic construct
VEGYRLFEKVW

SEQ ID NO: 11 - protein, 11 aa, synthetic construct
VSGWRIHEKIS

SEQ ID NO: 12 - protein, 11 aa, synthetic construct
VEGYRLFEKVW

SEQ ID NO: 13 - protein, 11 aa, synthetic construct
VEGYRLFERIW

SEQ ID NO: 14 - protein, 11 aa, synthetic construct
VEGYRLFERKW

SEQ ID NO: 15 - protein, 11 aa, synthetic construct
VEGYRLFNRKW

SEQ ID NO: 16 - protein, 11 aa, synthetic construct
VEGYRLFDRKL

SEQ ID NO: 17 - protein, 11 aa, synthetic construct
VEGYRLFDRKL

SEQ ID NO: 18 - protein, 11 aa, synthetic construct
VEGYRLFERVL

SEQ ID NO: 19 - protein, 11 aa, synthetic construct
VEGYRLFERKW

SEQ ID NO: 20 - protein, 11 aa, synthetic construct
VEGYRLFERIW

SEQ ID NO: 21 - protein, 11 aa, synthetic construct
VEGYRLFNEKS

SEQ ID NO: 22 - protein, 11 aa, synthetic construct
VEGYRLFNRKS

SEQ ID NO: 23 - protein, 11 aa, synthetic construct
VEGYRLFERKS

SEQ ID NO: 24 - protein, 11 aa, synthetic construct
VEGYRLFNKKS

SEQ ID NO: 25 - protein, 11 aa, synthetic construct
VEGYRLFERKL

SEQ ID NO: 26 - protein, 11 aa, synthetic construct
VEGYRLFNRVS

SEQ ID NO: 27 - protein, 11 aa, synthetic construct
VEGYRLFERKS

SEQ ID NO: 28 - protein, 11 aa, synthetic construct
VEGYRLFEKKL

SEQ ID NO: 29 - protein, 11 aa, synthetic construct
VEGYRLFNRKS

SEQ ID NO: 30 - protein, 11 aa, synthetic construct
VEGYRLFNRVG

SEQ ID NO: 31 - protein, 11 aa, synthetic construct
VEGYRLFNKEW

SEQ ID NO: 32 - protein, 11 aa, synthetic construct
VTGYRLFEEIL

SEQ ID NO: 33 - protein, 11 aa, synthetic construct
VDGWRLFDKKS

SEQ ID NO: 34 - protein, 11 aa, synthetic construct
VEGYRIFEKKW

SEQ ID NO: 35 - protein, 11 aa, synthetic construct
VEGYRLFDKVS

SEQ ID NO: 36 - protein, 11 aa, synthetic construct
VSGYRLFDRKW

SEQ ID NO: 37 - protein, 11 aa, synthetic construct
VEGYRLFERKS

SEQ ID NO: 38 - protein, 11 aa, synthetic construct
VEGYRLFEKVS

SEQ ID NO: 39 - protein, 11 aa, synthetic construct
VSGYRLFDKVS

SEQ ID NO: 40 - protein, 11 aa, synthetic construct
VDGWRLFDKKS

SEQ ID NO: 41 - protein, 11 aa, synthetic construct
VEGYRLFDKVS

SEQ ID NO: 42 - protein, 11 aa, synthetic construct
VEGYRLFDKVS

SEQ ID NO: 43 - protein, 11 aa, synthetic construct
VSGYRIFDKKS

SEQ ID NO: 44 - protein, 11 aa, synthetic construct
VSGYRLFDKKS

SEQ ID NO: 45 - protein, 11 aa, synthetic construct
VEGYRLFDRKS

SEQ ID NO: 46 - protein, 11 aa, synthetic construct
VSGYRLFDKKS

SEQ ID NO: 47 - protein, 11 aa, synthetic construct
VDGWRLFERKS

SEQ ID NO: 48 - protein, 11 aa, synthetic construct
VSGWRIFDKKS

SEQ ID NO: 49 - protein, 11 aa, synthetic construct
VSGYRLFDKKW

SEQ ID NO: 50 - protein, 11 aa, synthetic construct
VDGYRLFEKVS

SEQ ID NO: 51 - protein, 11 aa, synthetic construct
VSGYRLFDRKS

SEQ ID NO: 52 - protein, 11 aa, synthetic construct
VDGYRLFERKS

SEQ ID NO: 53 - protein, 11 aa, synthetic construct
VSGYRLFDKVS

SEQ ID NO: 54 - protein, 11 aa, synthetic construct
VDGWRLFDKKS

SEQ ID NO: 55 - protein, 11 aa, synthetic construct
VSGYRLFDKVS

SEQ ID NO: 56 - protein, 11 aa, synthetic construct
VEGYRLFEKIS

SEQ ID NO: 57 - protein, 11 aa, synthetic construct
VNGWRIFDKKS

SEQ ID NO: 58 - protein, 11 aa, synthetic construct
VSGYRIFERKW

SEQ ID NO: 59 - protein, 11 aa, synthetic construct
VSGYRIFEKKS

SEQ ID NO: 60 - protein, 11 aa, synthetic construct
VEGYRLFEKIS

SEQ ID NO: 61 - protein, 11 aa, synthetic construct
VEGWRLFDRKS

SEQ ID NO: 62 - protein, 11 aa, synthetic construct
VSGYRLFDRVW

SEQ ID NO: 63 - protein, 11 aa, synthetic construct
VSGYRIFEKKS

SEQ ID NO: 64 - protein, 11 aa, synthetic construct
VEGYRLFEKIS

SEQ ID NO: 65 - protein, 11 aa, synthetic construct
VSGYRLFDRKS

SEQ ID NO: 66 - protein, 11 aa, synthetic construct
VSGYRIFEKKW

SEQ ID NO: 67 - protein, 11 aa, synthetic construct
VEGWRIFERKW

SEQ ID NO: 68 - protein, 11 aa, synthetic construct
VSGYRLFDRKS

SEQ ID NO: 69 - protein, 11 aa, synthetic construct
VNGWRLFDKKS

SEQ ID NO: 70 - protein, 11 aa, synthetic construct
VEGYRLFERKS

SEQ ID NO: 71 - protein, 11 aa, synthetic construct
VEGWRLFDRVS

SEQ ID NO: 72 - protein, 11 aa, synthetic construct
VSGYRLFDRVS

SEQ ID NO: 73 - protein, 11 aa, synthetic construct
VSGWRIFDRKS

SEQ ID NO: 74 - protein, 11 aa, synthetic construct
VSGYRLFDKKW

SEQ ID NO: 75 - protein, 11 aa, synthetic construct
AEGYRLFDRKS

SEQ ID NO: 76 - protein, 11 aa, synthetic construct
AEGYRLFDRKS

SEQ ID NO: 77 - protein, 11 aa, synthetic construct
IEGYRLFDRKS

SEQ ID NO: 78 - protein, 11 aa, synthetic construct
AEGYRLFDRKS

SEQ ID NO: 79 - protein, 11 aa, synthetic construct
IEGYRLFDRKS

SEQ ID NO: 80 - protein, 11 aa, synthetic construct
VEPYKLFDRKS

SEQ ID NO: 81 - protein, 11 aa, synthetic construct
AEPYRIFDRKS

SEQ ID NO: 82 - protein, 11 aa, synthetic construct
AESYKLFDRKS

SEQ ID NO: 83 - protein, 11 aa, synthetic construct
VEGYHLFDRKS

SEQ ID NO: 84 - protein, 11 aa, synthetic construct
VEPYKLFDRKS

SEQ ID NO: 85 - protein, 11 aa, synthetic construct
AEGYHLFRSKS

SEQ ID NO: 86 - protein, 158 aa, synthetic construct
VFTLEDFVGDWEQTAAYNLDQVLEQGGVSSLLQNLAVSVTPIQRIVRSGENALKIDIHVIIPYEGLSADQMAQIEEVFKVVYPVDDHHFKVILPYGTLVIDGVTPNMLNYFGRPYEGIAVFDGKKITVTGTLWNGNKIIDERLITPDGSMLFRVTINS

SEQ ID NO: 87 - protein, 425 aa, synthetic construct
VFTLEDFVGDWEQTAAYNLDQVLEQGGVSSLLQNLAVSVTPIQRIVRSGENALKIDIHVIIPYEGLSADQMAQIEEVFKVVYPVDDHHFKVILPYGTLVIDGVTPNMLNYFGRPYEGIAVFDGKKITVTGTLWNGNKIIDERLITPDGSMLFRVTINSGSSGGGGSGGGGSGGQFVLTQPQSVSGSLGQTVSISCDRDSGNIEDYYVHWYRQHPGKAPTTVIYNDDQRPSGVPDRFSGSIDSTSNSASLTITGLLAEDEADYYCLSSDSSANVFGGGTKVVVESSGGGGSGGGGGGSSRSSQKQLVESGGGLVKPGASLTLTCKASGFSLSNKYYMSWVRQAPGKGLEWIAGIYVAISGTTHYASSVKGRFTISKPSSTTVTLQMTSLTAADTATYFCTNNLDLWGPGTLVTVSSGQAGHHHHHH

SEQ ID NO: 88 - protein, 278 aa, synthetic construct
AHHHHHHGSGDIVLTQTPSPVSAAVGGTVSINCQSSQSVYKNNRLSWYQQKPGQPPKFLIYDTSKLASGVPSRFSGSGSGTQFTLTISDLECDDAATYYCAGGYSNNIGAFGGGTEVVVKSSGGGGSGGGGGGSSRSSQSLEESRGRLVTPGGSLTLTCSVSGFSLSIYNMGWVRQAPGEGLEWIGVIGSSGNTYYASWAKGRFTISRNTNDNTVDLKITSPTTGDTATYFCARGFSSFDIWGPGTLVTVSSGGGGSGGGGSGGGGSVTGYRLFEEIL

SEQ ID NO: 89 - protein, 278 aa, synthetic construct
AHHHHHHGSGDIVLTQTPSPVSAAVGGTVSINCQSSQSVYKNNRLSWYQQKPGQPPKFLIYDTSKLASGVPSRFSGSGSGTQFTLTISDLECDDAATYYCAGGYSNNIGAFGGGTEVVVKSSGGGGSGGGGGGSSRSSQSLEESRGRLVTPGGSLTLTCSVSGFSLSIYNMGWVRQAPGEGLEWIGVIGSSGNTYYASWAKGRFTISRNTNDNTVDLKITSPTTGDTATYFCARGFSSFDIWGPGTLVTVSSGGGGSGGGGSGGGGSVEGYRLFDRKS

SEQ ID NO: 90 - protein, 192 aa, synthetic construct
PVPPGEDSKDVAAPHRQPLTSSERIDKQIRYILDGISALRKETCNKSNMCESSKEALAENNLNLPKMAEKDGCFQSGFNEETCLVKIITGLLEFEVYLEYLQNRFESSEEQARAVQMSTKVLIQFLQKKAKNLDAITTPDPTTNASLLTKLQAQNQWLQDMTTHLILRSFKEFLQSSLRALRQMAAHHHHHH

SEQ ID NO: 91 - protein, 284 aa, synthetic construct
VEGYRLFDRKSGGGGSGGGGSGGGGSQSALTQPSSVSKSLGQSVSITCSGSSSNVGYGNYVSWYQQVPGSAPKFLIYGATSRASGVPARFSGSRSGNTATLSISSLQAEDEADYYCASYDSSSYGVFGSGTTLTVLSSGGGGSGGGGGGSSRSSQVRLQESGPSLVKPSQTLSLTCTVSGFSLTNYPVGWVRQAPGKALEWLGGISSGGGTAYNPALKSRLSFTRDTSKNQVSLSLSSVTSEDTAVYYCTRGNGDYVLRYGADVWGRGLLVTVSSGSGHHHHHH

SEQ ID NO: 92 - protein, 433 aa, synthetic construct
VFTLEDFVGDWEQTAAYNLDQVLEQGGVSSLLQNLAVSVTPIQRIVRSGENALKIDIHVIIPYEGLSADQMAQIEEVFKVVYPVDDHHFKVILPYGTLVIDGVTPNMLNYFGRPYEGIAVFDGKKITVTGTLWNGNKIIDERLITPDGSMLFRVTINSGSSGGGGSGGGGSGGQAVLTQPSSVSKSLGQSVSITCSGSNIGSSAVGWYQQLPGSGLKTIIYSTSSRPSGVPDRFSGSKSGNTATLTISSLQAEDEADYYCATGDRGNYGGVFGSGTRLTVLSSGGGGSGGGGGGSSRSSQVQLQESGPSLVKPSQTLSLTCTVSGFSLTSYGVGWVRQAPGKTPEWLGGIDRDGDMSYNPALKSRLSITRDTSKSQVSLSLRSVATEDTAVYYCARSSYDSHYYGDYYDVDVWGRGLLVTVSSGQAGHHHHHH

SEQ ID NO: 93 - protein, 7 aa, synthetic construct
GGGSGGS

SEQ ID NO: 94 - protein, 9 aa, synthetic construct
GGGSGGGGS

SEQ ID NO: 95 - protein, 12 aa, synthetic construct
GGGSGGGSGGGS

SEQ ID NO: 96 - protein, 15 aa, synthetic construct
GGGGSGGGGSGGGGS

SEQ ID NO: 97 - protein, 7 aa, synthetic construct
AEAAAKA

SEQ ID NO: 98 - protein, 12 aa, synthetic construct
AEAAAKEAAAKA

SEQ ID NO: 99 - protein, 17 aa, synthetic construct
AEAAAKEAAAKEAAAKA

SEQ ID NO: 100 - protein, 7 aa, synthetic construct
GSSGGGS

SEQ ID NO: 101 - protein, 10 aa, synthetic construct
GSSGGGSGGS

SEQ ID NO: 102 - protein, 12 aa, synthetic construct
GSSGGGGSGGGS

SEQ ID NO: 103 - protein, 15 aa, synthetic construct
GSSGGGGSGGGGSGG

SEQ ID NO: 104 - protein, 24 aa, synthetic construct
NAEAAAKEAAAKALVPRGSGGGGS

SEQ ID NO: 105 - protein, 180 aa, synthetic construct
HHHHHVFTLEDFVGDWEQTAAYNLDQVLEQGGVSSLLQNLAVSVTPIQRIVRSGENALKIDIHVIIPYEGLSADQMAQIEEVFKVVYPVDDHHFKVILPYGTLVIDGVTPNMLNYFGRPYEGIAVFDGKKITVTGTLWNGNKIIDERLITPDGSMLFRVTINSGGGGSGGGGSGGGGSGC

SEQ ID NO: 106 - protein, 27 aa, synthetic construct
VEGYRLFDRKSGGGGSGGGGSGGGGSC